European Patent Specification EP 3 275 898 B1, published June 5, 2024. Title: Sema3A. Applicant: Osaka University. The sequence listing filed with the application follows.

SEQUENCE LISTING (16 sequences)

SEQ ID NO: 1 - protein, 771 aa, homo sapiens [sequence omitted]

SEQ ID NO: 2 - protein, 923 aa, Homo sapiens
MERGLPLLCAVLALVLAPAGAFRNDKCGDTIKIESPGYLTSPGYPHSYHPSEKCEWLIQAPDPYQRIMINFNPHFDLEDRDCKYDYVEVFDGENENGHFRGKFCGKIAPPPVVSSGPFLFIKFVSDYETHGAGFSIRYEIFKRGPECSQNYTTPSGVIKSPGFPEKYPNSLECTYIVFAPKMSEIILEFESFDLEPDSNPPGGMFCRYDRLEIWDGFPDVGPHIGRYCGQKTPGRIRSSSGILSMVFYTDSAIAKEGFSANYSVLQSSVSEDFKCMEALGMESGEIHSDQITASSQYSTNWSAERSRLNYPENGWTPGEDSYREWIQVDLGLLRFVTAVGTQGAISKETKKKYYVKTYKIDVSSNGEDWITIKEGNKPVLFQGNTNPTDVVVAVFPKPLITRFVRIKPATWETGISMRFEVYGCKITDYPCSGMLGMVSGLISDSQITSSNQGDRNWMPENIRLVTSRSGWALPPAPHSYINEWLQIDLGEEKIVRGIIIQGGKHRENKVFMRKFKIGYSNNGSDWKMIMDDSKRKAKSFEGNNNYDTPELRTFPALSTRFIRIYPERATHGGLGLRMELLGCEVEAPTAGPTTPNGNLVDECDDDQANCHSGTGDDFQLTGGTTVLATEKPTVIDSTIQSEFPTYGFNCEFGWGSHKTFCHWEHDNHVQLKWSVLTSKTGPIQDHTGDGNFIYSQADENQKGKVARLVSPVVYSQNSAHCMTFWYHMSGSHVGTLRVKLRYQKPEEYDQLVWMAIGHQGDHWKEGRVLLHKSLKLYQVIFEGEIGKGNLGGIAVDDISINNHISQEDCAKPADLDKKNPEIKIDETGSTPGYEGEGEGDKNISRKPGNVLKTLDPILITIIAMSALGVLLGAVCGVVLYCACWHNGMSERNLSALENYNFELVDGVKLKKDKLNTQSTYSEA

SEQ ID NO: 3 - protein, 1873 aa, Homo sapiens
MWAEAGLPRAGGGSQPPFRTFSASDWGLTHLVVHEQTGEVYVGAVNRIYKLSGNLTLLRAHVTGPVEDNEKCYPPPSVQSCPHGLGSTDNVNKLLLLDYAANRLLACGSASQGICQFLRLDDLFKLGEPHHRKEHYLSSVQEAGSMAGVLIAGPPGQGQAKLFVGTPIDGKSEYFPTLSSRRLMANEEDADMFGFVYQDEFVSSQLKIPSDTLSKFPAFDIYYVYSFRSEQFVYYLTLQLDTQLTSPDAAGEHFFTSKIVRLCVDDPKFYSYVEFPIGCEQAGVEYRLVQDAYLSRPGRALAHQLGLAEDEDVLFTVFAQGQKNRVKPPKESALCLFTLRAIKEKIKERIQSCYRGEGKLSLPWLLNKELGCINSPLQIDDDFCGQDFNQPLGGTVTIEGTPLFVDKDDGLTAVAAYDYRGRTVVFAGTRSGRIRKILVDLSNPGGRPALAYESVVAQEGSPILRDLVLSPNHQYLYAMTEKQVTRVPVESCVQYTSCELCLGSRDPHCGWCVLHSICSRRDACERADEPQRFAADLLQCVQLTVQPRNVSVTMSQVPLVLQAWNVPDLSAGVNCSFEDFTESESVLEDGRIHCRSPSAREVAPITRGQGDQRVVKLYLKSKETGKKFASVDFVFYNCSVHQSCLSCVNGSFPCHWCKYRHVCTHNVADCAFLEGRVNVSEDCPQILPSTQIYVPVGVVKPITLAARNLPQPQSGQRGYECLFHIPGSPARVTALRFNSSSLQCQNSSYSYEGNDVSDLPVNLSVVWNGNFVIDNPQNIQAHLYKCPALRESCGLCLKADPRFECGWCVAERRCSLRHHCAADTPASWMHARHGSSRCTDPKILKLSPETGPRQGGTRLTITGENLGLRFEDVRLGVRVGKVLCSPVESEYISAEQIVCEIGDASSVRAHDALVEVCVRDCSPHYRALSPKRFTFVTPTFYRVSPSRGPLSGGTWIGIEGSHLNAGSDVAVSVGGRPCSFSWRNSREIRCLTPPGQSPGSAPIIININRAQLTNPEVKYNYTEDPTILRIDPEWSINSGGTLLTVTGTNLATVREPRIRAKYGGIERENGCLVYNDTTMVCRAPSVANPVRSPPELGERPDELGFVMDNVRSLLVLNSTSFLYYPDPVLEPLSPTGLLELKPSSPLILKGRNLLPPAPGNSRLNYTVLIGSTPCTLTVSETQLLCEAPNLTGQHKVTVRAGGFEFSPGTLQVYSDSLLTLPAIVGIGGGGGLLLLVIVAVLIAYKRKSRDADRTLKRLQLQMDNLESRVALECKEAFAELQTDIHELTNDLDGAGIPFLDYRTYAMRVLFPGIEDHPVLKEMEVQANVEKSLTLFGQLLTKKHFLLTFIRTLEAQRSFSMRDRGNVASLIMTALQGEMEYATGVLKQLLSDLIEKNLESKNHPKLLLRRTESVAEKMLTNWFTFLLYKFLKECAGEPLFMLYCAIKQQMEKGPIDAITGEARYSLSEDKLIRQQIDYKTLTLNCVNPENENAPEVPVKGLDCDTVTQAKEKLLDAAYKGVPYSQRPKAADMDLEWRQGRMARIILQDEDVTTKIDNDWKRLNTLAHYQVTDGSSVALVPKQTSAYNISNSSTFTKSLSRYESMLRTASSPDSLRSRTPMITPDLESGTKLWHLVKNHDHLDQREGDRGSKMVSEIYLTRLLATKGTLQKFVDDLFETIFSTAHRGSALPLAIKYMFDFLDEQADKHQIHDADVRHTWKSNCLPLRFWVNVIKNPQFVFDIHKNSITDACLSVVAQTFMDSCSTSEHKLGKDSPSNKLLYAKDIPNYKSWVERYYADIAKMPAISDQDMSAYLAEQSRLHLSQFNSMSALHEIYSYITKYKDEILAALEKDEQARRQRLRSKLEQVVDTMALSS

SEQ ID NO: 4 - DNA, 2316 bp, Homo sapiens
atgggctggttaactaggattgtctgtcttttctggggagtattacttacagcaagagcaaactatcagaatgggaagaacaatgtgccaaggctgaaattatcctacaaagaaatgttggaatccaacaatgtgatcactttcaatggcttggccaacagctccagttatcataccttccttttggatgaggaacggagtaggctgtatgttggagcaaaggatcacatattttcattcgacctggttaatatcaaggattttcaaaagattgtgtggccagtatcttacaccagaagagatgaatgcaagtgggctggaaaagacatcctgaaagaatgtgctaatttcatcaaggtacttaaggcatataatcagactcacttgtacgcctgtggaacgggggcttttcatccaatttgcacctacattgaaattggacatcatcctgaggacaatatttttaagctggagaactcacattttgaaaacggccgtgggaagagtccatatgaccctaagctgctgacagcatcccttttaatagatggagaattatactctggaactgcagctgattttatggggcgagactttgctatcttccgaactcttgggcaccaccacccaatcaggacagagcagcatgattccaggtggctcaatgatccaaagttcattagtgcccacctcatctcagagagtgacaatcctgaagatgacaaagtatactttttcttccgtgaaaatgcaatagatggagaacactctggaaaagctactcacgctagaataggtcagatatgcaagaatgactttggagggcacagaagtctggtgaataaatggacaacattcctcaaagctcgtctgatttgctcagtgccaggtccaaatggcattgacactcattttgatgaactgcaggatgtattcctaatgaactttaaagatcctaaaaatccagttgtatatggagtgtttacgacttccagtaacattttcaagggatcagccgtgtgtatgtatagcatgagtgatgtgagaagggtgttccttggtccatatgcccacagggatggacccaactatcaatgggtgccttatcaaggaagagtcccctatccacggccaggaacttgtcccagcaaaacatttggtggttttgactctacaaaggaccttcctgatgatgttataacctttgcaagaagtcatccagccatgtacaatccagtgtttcctatgaacaatcgcccaatagtgatcaaaacggatgtaaattatcaatttacacaaattgtcgtagaccgagtggatgcagaagatggacagtatgatgttatgtttatcggaacagatgttgggaccgttcttaaagtagtttcaattcctaaggagacttggtatgatttagaagaggttctgctggaagaaatgacagtttttcgggaaccgactgctatttcagcaatggagctttccactaagcagcaacaactatatattggttcaacggctggggttgcccagctccctttacaccggtgtgatatttacgggaaagcgtgtgctgagtgttgcctcgcccgagacccttactgtgcttgggatggttctgcatgttctcgctattttcccactgcaaagagacgcacaagacgacaagatataagaaatggagacccactgactcactgttcagacttacaccatgataatcaccatggccacagccctgaagagagaatcatctatggtgtagagaatagtagcacatttttggaatgcagtccgaagtcgcagagagcgctggtctattggcaattccagaggcgaaatgaagagcgaaaagaagagatcagagtggatgatcatatcatcaggacagatcaaggccttctgctacgtagtctacaacagaaggattcaggcaattacctctgccatgcggtggaacatgggttcatacaaactcttcttaaggtaaccctggaagtcattgacacagagcatttggaagaacttcttcataaagatgatgatggagatggctctaagaccaaagaaatgtccaatagcatgacacctagccagaaggtctggtacagagacttcatgcagctcatcaaccaccccaatctcaacacaatggatgagttctgtgaacaagtttggaaaagggaccgaaaacaacgtcggcaaaggccaggacataccccagggaacagtaacaaatggaagcacttacaagaaaataagaaaggtagaaacaggaggacccacgaatttgagagggcacccaggagtgtctga

SEQ ID NO: 5 - DNA, 2772 bp, Homo sapiens
atggagagggggctgccgctcctctgcgccgtgctcgccctcgtcctcgccccggccggcgcttttcgcaacgataaatgtggcgatactataaaaattgaaagccccgggtaccttacatctcctggttatcctcattcttatcacccaagtgaaaaatgcgaatggctgattcaggctccggacccataccagagaattatgatcaacttcaaccctcacttcgatttggaggacagagactgcaagtatgactacgtggaagtcttcgatggagaaaatgaaaatggacattttaggggaaagttctgtggaaagatagcccctcctcctgttgtgtcttcagggccatttctttttatcaaatttgtctctgactacgaaacacatggtgcaggattttccatacgttatgaaattttcaagagaggtcctgaatgttcccagaactacacaacacctagtggagtgataaagtcccccggattccctgaaaaatatcccaacagccttgaatgcacttatattgtctttgcgccaaagatgtcagagattatcctggaatttgaaagctttgacctggagcctgactcaaatcctccaggggggatgttctgtcgctacgaccggctagaaatctgggatggattccctgatgttggccctcacattgggcgttactgtggacagaaaacaccaggtcgaatccgatcctcatcgggcattctctccatggttttttacaccgacagcgcgatagcaaaagaaggtttctcagcaaactacagtgtcttgcagagcagtgtctcagaagatttcaaatgtatggaagctctgggcatggaatcaggagaaattcattctgaccagatcacagcttcttcccagtatagcaccaactggtctgcagagcgctcccgcctgaactaccctgagaatgggtggactcccggagaggattcctaccgagagtggatacaggtagacttgggccttctgcgctttgtcacggctgtcgggacacagggcgccatttcaaaagaaaccaagaagaaatattatgtcaagacttacaagatcgacgttagctccaacggggaagactggatcaccataaaagaaggaaacaaacctgttctctttcagggaaacaccaaccccacagatgttgtggttgcagtattccccaaaccactgataactcgatttgtccgaatcaagcctgcaacttgggaaactggcatatctatgagatttgaagtatacggttgcaagataacagattatccttgctctggaatgttgggtatggtgtctggacttatttctgactcccagatcacatcatccaaccaaggggacagaaactggatgcctgaaaacatccgcctggtaaccagtcgctctggctgggcacttccacccgcacctcattcctacatcaatgagtggctccaaatagacctgggggaggagaagatcgtgaggggcatcatcattcagggtgggaagcaccgagagaacaaggtgttcatgaggaagttcaagatcgggtacagcaacaacggctcggactggaagatgatcatggatgacagcaaacgcaaggcgaagtcttttgagggcaacaacaactatgatacacctgagctgcggacttttccagctctctccacgcgattcatcaggatctaccccgagagagccactcatggcggactggggctcagaatggagctgctgggctgtgaagtggaagcccctacagctggaccgaccactcccaacgggaacttggtggatgaatgtgatgacgaccaggccaactgccacagtggaacaggtgatgacttccagctcacaggtggcaccactgtgctggccacagaaaagcccacggtcatagacagcaccatacaatcagagtttccaacatatggttttaactgtgaatttggctggggctctcacaagaccttctgccactgggaacatgacaatcacgtgcagctcaagtggagtgtgttgaccagcaagacgggacccattcaggatcacacaggagatggcaacttcatctattcccaagctgacgaaaatcagaagggcaaagtggctcgcctggtgagccctgtggtttattcccagaactctgcccactgcatgaccttctggtatcacatgtctgggtcccacgtcggcacactcagggtcaaactgcgctaccagaagccagaggagtacgatcagctggtctggatggccattggacaccaaggtgaccactggaaggaagggcgtgtcttgctccacaagtctctgaaactttatcaggtgattttcgagggcgaaatcggaaaaggaaaccttggtgggattgctgtggatgacattagtattaataaccacatttcacaagaagattgtgcaaaaccagcagacctggataaaaagaacccagaaattaaaattgatgaaacagggagcacgccaggatacgaaggtgaaggagaaggtgacaagaacatctccaggaagccaggcaatgtgttgaagaccttagaccccatcctcatcaccatcatagccatgagtgccctgggggtcctcctgggggctgtctgtggggtcgtgctgtactgtgcctgttggcataatgggatgtcagaaagaaacttgtctgccctggagaactataactttgaacttgtggatggtgtgaagttgaaaaaagacaaactgaatacacagagtacttattcggaggcatga

SEQ ID NO: 6 - DNA, 5622 bp, Homo sapiens
atgtgggctgaggcaggcttgcccagggcaggcgggggttcacagccccccttccgcaccttctcggccagcgactggggcctcacccacctagtggtgcatgagcagacaggcgaggtgtatgtgggcgcagtgaaccgcatctataagctgtcggggaacctgacactgctgcgggcccacgtcacgggccctgtggaggacaacgagaagtgctacccgccgcccagcgtgcagtcctgcccccacggcctgggcagtactgacaacgtcaacaagctgctgctgctggactatgccgctaaccgcctgctggcctgtggcagcgcctcccagggcatctgccagttcctgcgtctggacgatctcttcaaactgggtgagccacaccaccgtaaggagcactacctgtccagcgtgcaggaggcaggcagcatggcgggcgtgctcattgccgggccaccgggccagggccaggccaagctcttcgtgggcacacccatcgatggcaagtccgagtacttccccacactgtccagccgtcggctcatggccaacgaggaggatgccgacatgttcggcttcgtgtaccaggatgagtttgtgtcatcacagctcaagatcccttcggacacgctgtccaagttcccggcctttgacatctactatgtgtacagcttccgcagcgagcagtttgtctactacctcacgctgcagctagacacacagctgacctcgcctgatgccgccggcgagcacttcttcacgtccaagatcgtgcggctctgtgtggacgaccccaaattctactcgtacgttgagttccccattggctgcgagcaggcgggtgtggagtaccgcctggtgcaggatgcctacctgagccggcccggccgtgccctggcccaccagctgggcctggctgaggacgaggacgtgctgttcactgtgttcgcccagggccagaagaaccgcgtgaagccaccaaaggagtcagcactgtgcctgttcacgctcagggccatcaaggagaagattaaggagcgcatccagtcctgctaccgtggtgagggcaagctctccctgccgtggctgctcaacaaggagctgggctgcatcaactcgcccctgcagatcgatgacgacttctgcgggcaggacttcaaccagcccctggggggcacagtcaccattgaggggacgcccctgttcgtggacaaggatgatggcctgaccgccgtggctgcctatgactatcggggccgcactgtggtattcgccggcacgcgaagtggccgcatccgcaagatcctggtggacctctcaaaccccggtggccggcctgccctggcctacgagagcgtcgtggcccaggagggcagccccatcctgcgagacctcgtcctcagccccaaccaccagtacctctacgccatgaccgagaagcaggtgacgcgggtgcctgtggagagctgtgtgcagtacacgtcctgtgagctgtgtctggggtcacgggacccccactgtggctggtgtgtcctgcacagcatctgctcgcggcgggacgcctgtgagcgagcagacgagccccagcgctttgctgcggacctgctgcagtgtgtgcagctgactgtgcagccccgcaatgtgtctgtcaccatgtcccaggtcccacttgtgctgcaggcctggaacgtgcctgacctctcagctggcgtcaactgctccttcgaggacttcacggaatctgagagcgtcctggaggatggccggatccactgccgctcaccctccgcccgggaggtggcgcccatcacgcggggccagggagaccagcgggtggtgaaactctacctaaagtccaaggagacagggaagaagtttgcgtctgtggacttcgtcttctacaactgcagcgtccaccagtcctgcctgtcctgtgtcaacggctcctttccctgccactggtgcaaataccgccacgtgtgcacacacaacgtggctgactgcgccttcctggagggccgtgtcaacgtgtctgaggactgcccacagatcctgccctccacgcagatctacgtgccagtgggagtggtaaaacccatcaccctggccgcacggaacctgccacagccacagtcaggccagcgtggatatgagtgcctcttccacatcccgggcagcccggcccgtgtcaccgccctgcgcttcaacagctccagcctgcagtgccagaattcctcgtactcctacgaggggaacgatgtcagcgacctgccagtgaacctgtcagtcgtgtggaacggcaactttgtcattgacaacccacagaacatccaggcgcacctctacaagtgcccggccctgcgcgagagctgcggcctctgcctcaaggccgacccgcgcttcgagtgcggatggtgcgtggccgagcgccgctgctccctgcgacaccactgcgctgccgacacacctgcatcgtggatgcacgcgcgtcacggcagcagtcgctgcaccgaccccaagatcctcaagctgtcccccgagacgggcccgaggcagggcggcacgcggctcactatcacaggcgagaacctgggcctgcgattcgaagacgtgcgtctgggcgtgcgcgtgggcaaggtgctgtgcagccctgtggagagcgagtacatcagtgcggagcagatcgtctgtgagatcggggacgccagctccgtgcgtgcccatgacgccctggtggaggtgtgtgtgcgggactgctcaccacactaccgcgccctgtcacccaagcgcttcaccttcgtgacaccaaccttctaccgtgtgagcccctcccgtgggcctctgtcagggggcacctggattggcatcgagggaagccacctgaacgcaggcagtgatgtggctgtgtcggtcggtggccggccctgctccttctcctggaggaactcccgtgagatccggtgcctgacaccccccgggcagagccctggcagcgctcccatcatcatcaacatcaaccgcgcccagctcaccaaccctgaggtgaagtacaactacaccgaggaccccaccatcctgaggatcgaccccgagtggagcatcaacagcggtgggaccctcctgacggtcacaggcaccaacctggccactgtccgtgaaccccgaatccgggccaagtatggaggcattgagagggagaacggctgcctggtgtacaatgacaccaccatggtatgccgcgccccgtctgtggccaaccctgtgcgcagcccaccagagctgggggagcggccggatgagctgggcttcgtcatggacaacgtgcgctccctgcttgtgctcaactccacctccttcctctactaccctgaccccgtactggagccactcagccccactggcctgctggagctgaagcccagctccccactcatcctcaagggccggaacctcttgccacctgcacccggcaactcccgactcaactacacggtgctcatcggctccacaccctgtaccctcaccgtgtcggagacgcaactgctgtgcgaggcgcccaacctcactgggcagcacaaggtcacggtgcgggcaggtggcttcgagttctcgccagggacactgcaggtgtactcggacagcctgctgacgctgcctgccattgtgggcattggcggaggcgggggtctcctgctgctggtcatcgtggctgtgctcatcgcctacaagcgcaagtcacgagatgctgaccgcacactcaagcggctgcagctccagatggacaacctggagtcccgcgtggccctcgaatgcaaggaagcctttgcagagctgcagacagacatccacgagctgaccaatgacctggacggtgccggcatccccttccttgactaccggacatatgccatgcgggtgctctttcctgggatcgaggaccaccctgtgctcaaggagatggaggtgcaggccaatgtggagaagtcgctgacactgttcgggcagctgctgaccaagaagcacttcctgctgaccttcatccgcacgctggaggcacagcgcagcttctccatgcgcgaccgcgggaatgtggcctcgctcatcatgacggccctgcagggcgagatggaatacgccacaggcgtgctcaagcagctgctttccgacctcatcgagaagaacctggagagcaagaaccaccccaagctgctactgcgccggactgagtcggtggcagagaagatgctaactaactggttcaccttcctcttgtataagttcctcaaggagtgcgctggggagccgctgttcatgctgtactgcgccatcaagcagcagatggagaagggccccattgacgccatcacgggtgaggcacgctactccctgagtgaggacaagctcatccggcagcagattgactacaagacactgaccctgaactgtgtgaaccctgagaatgagaatgcacctgaggtgccggtgaaggggctggactgtgacacggtcacccaggccaaggagaagctgctggacgctgcctacaagggcgtgccctactcccagcggcccaaggccgcggacatggacctggagtggcgccagggccgcatggcgcgcatcatcctgcaggacgaggacgtcaccaccaagattgacaacgattggaagaggctgaacacactggctcactaccaggtgacagacgggtcctcggtggcactggtgcccaagcagacgtccgcctacaacatctccaactcctccaccttcaccaagtccctcagcagatacgagagcatgctgcgcacggccagcagccccgacagcctgcgctcgcgcacgcccatgatcacgcccgacctggagagcggcaccaagctgtggcacctggtgaagaaccacgaccacctggaccagcgtgagggtgaccgcggcagcaagatggtctcggagatctacttgacacggctactggccaccaagggcacactgcagaagtttgtggacgacctgtttgagaccatcttcagcacggcacaccggggctcagccctgccgctggccatcaagtacatgttcgacttcctggatgagcaggccgacaagcaccagatccacgatgctgacgtgcgccacacctggaagagcaactgcctgcccctgcgcttctgggtgaacgtgatcaagaacccacagtttgtgttcgacattcacaagaacagcatcacggacgcctgcttgtcggtggtggcccagaccttcatggactcctgctccacctctgagcacaagctgggcaaggactcaccctccaacaagctgctctacgccaaggacatccccaactacaagagctgggtggagaggtactatgcagacatcgccaagatgccagccatcagcgaccaggacatgagtgcgtatctggctgagcagtcccgcctgcacctgagccagttcaacagcatgagcgccttgcacgagatctactcctacatcaccaagtacaaggatgagatcctggcagccctggagaaggatgagcaggcgcggcggcagcggctgcggagcaagctggagcaggtggtggacacgatggccctgagcagctga

SEQ ID NO: 7 - protein, 223 aa, Homo sapiens
TCPPCPAPELLGGPSVFLFPPKPKDTLMISRTPEVTCVVVDVSHEDPEVKFNWYVDGVEVHNAKTKPREEQYNSTYRVVSVLTVLHQDWLNGKEYKCKVSNKALPAPIEKTISKAKGQPREPQVYTLPPSRDELTKNQVSLTCLVKGFYPSDIAVEWESNGQPENNYKTTPPVLDSDGPFFLYSKLTVDKSRWQQGNVFSCSVMHEALHNHYTQKSLSLSPGK

SEQ ID NO: 8 - protein, 221 aa, Homo sapiens
CPPCPAPPVAGPSVFLFPPKPKDTLMISRTPEVTCVVVDVSHEDPEVQFNWYVDGVEVHNAKTKPREEQFNSTFRVVSVLTVVHQDWLNGKEYKCKVSNKGLPAPIEKTISKTKGQPREPQVYTLPPSREEMTKNQVSLTCLVKGFYPSDISVEWESNGQPENNYKTTPPMLDSDGSFFLYSKLTVDKSRWQQGNVFSCSVMHEALHNHYTQKSLSLSPGK

SEQ ID NO: 9 - protein, 222 aa, Homo sapiens
CPRCPAPELLGGPSVFLFPPKPKDTLMISRTPEVTCVVVDVSHEDPEVQFKWYVDGVEVHNAKTKPREEQYNSTFRVVSVLTVLHQDWLNGKEYKCKVSNKALPAPIEKTISKTKGQPREPQVYTLPPSREEMTKNQVSLTCLVKGFYPSDIAVEWESSGQPENNYNTTPPMLDSDGSFFLYSKLTVDKSRWQQGNIFSCSVMHEALHNRFTQKSLSLSPGK

SEQ ID NO: 10 - protein, 222 aa, Homo sapiens
CPSCPAPEFLGGPSVFLFPPKPKDTLMISRTPEVTCVVVDVSQEDPEVQFNWYVDGVEVHNAKTKPREEQFNSTYRVVSVLTVLHQDWLNGKEYKCKVSNKGLPSSIEKTISKAKGQPREPQVYTLPPSQEEMTKNQVSLTCLVKGFYPSDIAVEWESNGQPENNYKTTPPVLDSDGSFFLYSRLTVDKSRWQEGNVFSCSVMHEALHNHYTQKSLSLSLGK

SEQ ID NO: 11 - protein, 923 aa, Mus musculus
MERGLPLLCATLALALALAGAFRSDKCGGTIKIENPGYLTSPGYPHSYHPSEKCEWLIQAPEPYQRIMINFNPHFDLEDRDCKYDYVEVIDGENEGGRLWGKFCGKIAPSPVVSSGPFLFIKFVSDYETHGAGFSIRYEIFKRGPECSQNYTAPTGVIKSPGFPEKYPNSLECTYIIFAPKMSEIILEFESFDLEQDSNPPGGMFCRYDRLEIWDGFPEVGPHIGRYCGQKTPGRIRSSSGVLSMVFYTDSAIAKEGFSANYSVLQSSISEDFKCMEALGMESGEIHSDQITASSQYGTNWSVERSRLNYPENGWTPGEDSYKEWIQVDLGLLRFVTAVGTQGAISKETKKKYYVKTYRVDISSNGEDWISLKEGNKAIIFQGNTNPTDVVLGVFSKPLITRFVRIKPVSWETGISMRFEVYGCKITDYPCSGMLGMVSGLISDSQITASNQADRNWMPENIRLVTSRTGWALPPSPHPYTNEWLQVDLGDEKIVRGVIIQGGKHRENKVFMRKFKIAYSNNGSDWKTIMDDSKRKAKSFEGNNNYDTPELRTFSPLSTRFIRIYPERATHSGLGLRMELLGCEVEAPTAGPTTPNGNPVDECDDDQANCHSGTGDDFQLTGGTTVLATEKPTIIDSTIQSEFPTYGFNCEFGWGSHKTFCHWEHDSHAQLRWSVLTSKTGPIQDHTGDGNFIYSQADENQKGKVARLVSPVVYSQSSAHCMTFWYHMSGSHVGTLRVKLRYQKPEEYDQLVWMVVGHQGDHWKEGRVLLHKSLKLYQVIFEGEIGKGNLGGIAVDDISINNHISQEDCAKPTDLDKKNTEIKIDETGSTPGYEGEGEGDKNISRKPGNVLKTLDPILITIIAMSALGVLLGAVCGVVLYCACWHNGMSERNLSALENYNFELVDGVKLKKDKLNPQSNYSEA

SEQ ID NO: 12 - protein, 19 aa, Homo sapiens
NYQWVPYQGRVPYPRPGTC

SEQ ID NO: 13 - DNA, 23 bp, Artificial
  PCR primer
acaaacgagaaaccagtttcacc

SEQ ID NO: 14 - DNA, 23 bp, Artificial
  PCR primer
ccagcaatataaagtgtgtctcg

SEQ ID NO: 15 - DNA, 25 bp, Artificial
  PCR primer
caatatccggtttttagaggacgcc

SEQ ID NO: 16 - DNA, 25 bp, Artificial
  PCR primer
cctgctgtctggacctccacgtcag